European Patent Specification EP 4 181 907 B1, published September 3, 2025. Title: METHOD OF TREATMENT OF CONGENITAL MYASTHENIC SYNDROME USING DOK7 GENE OR POLYPEPTIDE. Applicant: Oxford University Innovation Limited. The sequence listing filed with the application follows.

SEQUENCE LISTING (12 sequences)

SEQ ID NO: 1 - DNA, 1449 bp, Homo sapiens
atggagccctggcctctcctcctgctctttagcctttgctcagctggcctcgtcctgggctccgaacatgagacccgtctggtggcaaagctatttaaagactacagcagcgtggtgcggccagtggaagaccaccgccaggtcgtggaggtcaccgtgggcctgcagctgatacagctcatcaatgtggatgaagtaaatcagatcgtgacaaccaatgtgcgtctgaaacagggtgacatggtagatctgccacgccccagctgcgtgactttgggagttcctttgttttctcatctgcagaatgagcaatgggtggattacaacctaaaatggaatccagatgactatggcggtgtgaaaaaaattcacattccttcagaaaagatctggcgcccagaccttgttctctataacaatgcagatggtgactttgctattgtcaagttcaccaaagtgctcctgcagtacactggccacatcacgtggacacctccagccatctttaaaagctactgtgagatcatcgtcacccactttccctttgatgaacagaactgcagcatgaagctgggcacctggacctacgacggctctgtcgtggccatcaacccggaaagcgaccagccagacctgagcaacttcatggagagcggggagtgggtgatcaaggagtcccggggctggaagcactccgtgacctattcctgctgccccgacaccccctacctggacatcacctaccacttcgtcatgcagcgcctgcccctctacttcatcgtcaacgtcatcatcccctgcctgctcttctccttcttaactggcctggtattctacctgcccacagactcaggggagaagatgactctgagcatctctgtcttactgtctttgactgtgttccttctggtcatcgtggagctgatcccctccacgtccagtgctgtgcccttgattggaaaatacatgctgttcaccatggtgttcgtcattgcctccatcatcatcactgtcatcgtcatcaacacacaccaccgctcacccagcacccatgtcatgcccaactgggtgcggaaggtttttatcgacactatcccaaatatcatgtttttctccacaatgaaaagaccatccagagaaaagcaagacaaaaagatttttacagaagacattgatatctctgacatttctggaaagccagggcctccacccatgggcttccactctcccctgatcaaacaccccgaggtgaaaagtgccatcgagggcatcaagtacatcgcagagaccatgaagtcagaccaggagtctaacaatgcggcggcagagtggaagtacgttgcaatggtgatggaccacatactcctcggagtcttcatgcttgtttgcatcatcggaaccctagccgtgtttgcaggtcgactcattgaattaaatcagcaaggatga

SEQ ID NO: 2 - protein, 482 aa, Homo sapiens
MEPWPLLLLFSLCSAGLVLGSEHETRLVAKLFKDYSSVVRPVEDHRQVVEVTVGLQLIQLINVDEVNQIVTTNVRLKQGDMVDLPRPSCVTLGVPLFSHLQNEQWVDYNLKWNPDDYGGVKKIHIPSEKIWRPDLVLYNNADGDFAIVKFTKVLLQYTGHITWTPPAIFKSYCEIIVTHFPFDEQNCSMKLGTWTYDGSVVAINPESDQPDLSNFMESGEWVIKESRGWKHSVTYSCCPDTPYLDITYHFVMQRLPLYFIVNVIIPCLLFSFLTGLVFYLPTDSGEKMTLSISVLLSLTVFLLVIVELIPSTSSAVPLIGKYMLFTMVFVIASIIITVIVINTHHRSPSTHVMPNWVRKVFIDTIPNIMFFSTMKRPSREKQDKKIFTEDIDISDISGKPGPPPMGFHSPLIKHPEVKSAIEGIKYIAETMKSDQESNNAAAEWKYVAMVMDHILLGVFMLVCIIGTLAVFAGRLIELNQQG

SEQ ID NO: 3 - DNA, 1506 bp, Homo sapiens
atgaccccaggggctctgctgatgctgctgggggcgctgggggcgccgctcgccccaggcgtccgcggctcggaggcggagggtcgactccgggagaaacttttctctggctatgatagctccgtgcggccagcgcgggaggtgggagaccgtgtcagggtcagcgttggtctcatcctggcgcaactcatcagcctgaacgagaaggatgaagagatgagcacaaaggtgtacttagacctggagtggactgactacaggctgagctgggaccctgcggagcacgacggcatcgattcgctccgcatcacggcggaatccgtgtggctccctgacgtggtgctactgaacaacaatgatgggaattttgacgtggctctggacattagcgtcgtggtgtcctccgacggctccgtgcgttggcaacccccgggcatctatcgcagcagctgcagcatccaggtcacctacttccccttcgactggcagaattgcactatggtgttcagctcctacagctacgacagctcggaggtcagcctgcagacaggcctgggtcctgacgggcaagggcatcaggaaatccacattcatgaagggactttcattgagaatggccagtgggagattatccacaagccctctcggctaatccagcctccaggcgatcctaggggagggagggaaggacagcgccaggaagtcatcttctacctcatcatccgccgcaagcctctcttctacctggtcaacgtcattgccccatgcatcctcatcactcttctggccatcttcgtcttctacctgccaccagatgcaggagagaagatggggctctcaatctttgccctgctgacccttactgtgttcctgctgctgctggctgacaaagtacctgagacctcactatcagtacccattattatcaagtacctcatgtttaccatggtcctcgtcaccttctcagtcatccttagtgtcgtggttctcaacctgcaccaccgctcaccccacacccaccaaatgcccctttgggtccgtcagatcttcattcacaaacttccgctgtacctgcgtctaaaaaggcccaaacccgagagagacctgatgccggagccccctcactgttcttctccaggaagtggctggggtcggggaacagatgaatatttcatccggaagccgccaagtgattttctcttccccaaacccaataggttccagcctgaactgtctgcccctgatctgcggcgatttatcgatggtccaaaccgggctgtggccctgcttccggagctacgggaggtcgtctcctctatcagctacatcgctcgacagctgcaggaacaggaggaccacgatgcgctgaaggaggactggcagtttgtggccatggtagtggaccgcctcttcctgtggactttcatcatcttcaccagcgttgggaccctagtcatcttcctggacgccacgtaccacttgccccctccagacccctttccttga

SEQ ID NO: 4 - protein, 501 aa, Homo sapiens
MTPGALLMLLGALGAPLAPGVRGSEAEGRLREKLFSGYDSSVRPAREVGDRVRVSVGLILAQLISLNEKDEEMSTKVYLDLEWTDYRLSWDPAEHDGIDSLRITAESVWLPDVVLLNNNDGNFDVALDISVVVSSDGSVRWQPPGIYRSSCSIQVTYFPFDWQNCTMVFSSYSYDSSEVSLQTGLGPDGQGHQEIHIHEGTFIENGQWEIIHKPSRLIQPPGDPRGGREGQRQEVIFYLIIRRKPLFYLVNVIAPCILITLLAIFVFYLPPDAGEKMGLSIFALLTLTVFLLLLADKVPETSLSVPIIIKYLMFTMVLVTFSVILSVVVLNLHHRSPHTHQMPLWVRQIFIHKLPLYLRLKRPKPERDLMPEPPHCSSPGSGWGRGTDEYFIRKPPSDFLFPKPNRFQPELSAPDLRRFIDGPNRAVALLPELREVVSSISYIARQLQEQEDHDALKEDWQFVAMVVDRLFLWTFIIFTSVGTLVIFLDATYHLPPPDPFP

SEQ ID NO: 5 - DNA, 1554 bp, Homo sapiens
atggaggggccagtgctgacactggggctgctggctgccctggcggtgtgtggcagctgggggctgaacgaggaggagcggctgatccggcacctgtttcaagagaagggctacaacaaggagctccggcccgtggcacacaaagaggagagtgtggacgttgccctggccctcacactctccaacctcatctccctgaaagaagttgaggagaccctcactaccaatgtgtggatagagcacggctggacagacaaccggctgaagtggaatgctgaagaatttggaaacatcagtgtcctgcgcctccccccggacatggtgtggctcccagagattgtgctggagaacaacaatgacggctccttccagatctcctactcctgcaacgtgcttgtctaccactacggcttcgtgtactggctgccacctgccatcttccgctcctcctgccccatctctgtcacctatttccccttcgactggcagaactgctccctcaagttcagttccctcaagtatacggccaaagagatcaccctgagcctgaaacaggatgccaaggagaaccgcacctaccccgtggagtggatcatcattgatcctgaaggcttcacagagaacggggagtgggagatagtccaccggccggccagggtcaacgtggaccccagagcccctctggacagccccagccgccaggacatcaccttctacctcatcatccgccgcaagcccctcttctacatcatcaacatcctggtgccctgcgtgctcatctccttcatggtcaacctggtcttctacctaccggctgacagtggtgagaagacatcagtggccatctcggtgctcctggctcagtctgtcttcctgctgctcatctccaagcgtctgcctgccacatccatggccatcccccttatcggcaagttcctgctcttcggcatggtgctggtcaccatggttgtggtgatctgtgtcatcgtgctcaacatccacttccgaacacccagcacccatgtgctgtctgagggggtcaagaagctcttcctggagaccctgccggagctcctgcacatgtcccgcccagcagaggatggacccagccctggggccctggtgcggaggagcagctccctgggatacatctccaaggccgaggagtacttcctgctcaagtcccgcagtgacctcatgttcgagaagcagtcagagcggcatgggctggccaggcgcctcaccactgcacgccggcccccagcaagctctgagcaggcccagcaggaactcttcaatgagctgaagccagctgtggatggggcaaacttcattgttaaccacatgagggaccagaacaattacaatgaggagaaagacagctggaaccgagtggcccgcacagtggaccgcctctgcctgtttgtggtgacgcctgtcatggtggtgggcacagcctggatcttcctgcagggcgtttacaaccagccaccaccccagccttttcctggggacccctactcctacaacgtgcaggacaagcgcttcatctag

SEQ ID NO: 6 - protein, 517 aa, Homo sapiens
MEGPVLTLGLLAALAVCGSWGLNEEERLIRHLFQEKGYNKELRPVAHKEESVDVALALTLSNLISLKEVEETLTTNVWIEHGWTDNRLKWNAEEFGNISVLRLPPDMVWLPEIVLENNNDGSFQISYSCNVLVYHYGFVYWLPPAIFRSSCPISVTYFPFDWQNCSLKFSSLKYTAKEITLSLKQDAKENRTYPVEWIIIDPEGFTENGEWEIVHRPARVNVDPRAPLDSPSRQDITFYLIIRRKPLFYIINILVPCVLISFMVNLVFYLPADSGEKTSVAISVLLAQSVFLLLISKRLPATSMAIPLIGKFLLFGMVLVTMVVVICVIVLNIHFRTPSTHVLSEGVKKLFLETLPELLHMSRPAEDGPSPGALVRRSSSLGYISKAEEYFLLKSRSDLMFEKQSERHGLARRLTTARRPPASSEQAQQELFNELKPAVDGANFIVNHMRDQNNYNEEKDSWNRVARTVDRLCLFVVTPVMVVGTAWIFLQGVYNQPPPQPFPGDPYSYNVQDKRFI

SEQ ID NO: 7 - DNA, 1482 bp, Homo sapiens
atggcaagggctccgcttggggtcctgctcctcttggggcttctcggcaggggtgtggggaagaacgaggaactgcgtctttatcaccatctcttcaacaactatgacccaggaagccggccagtgcgggagcctgaggatactgtcaccatcagcctcaaggtcaccctgacgaatctcatctcactgaatgaaaaagaggagactctcaccactagcgtctggattggaatcgattggcaggattaccgactcaactacagcaaggacgactttgggggtatagaaaccctgcgagtcccttcagaactcgtgtggctgccagagattgtgctggaaaacaatattgatggccagttcggagtggcctacgacgccaacgtgctcgtctacgagggcggctccgtgacgtggctgcctccggccatctaccgcagcgtctgcgcagtggaggtcacctacttccccttcgattggcagaactgttcgcttattttccgctctcagacgtacaatgccgaagaggtggagttcacttttgccgtagacaacgacggcaagaccatcaacaagatcgacatcgacacagaggcctatactgagaacggcgagtgggccatcgacttctgcccgggggtgatccgccgccaccacggtggcgccaccgacggcccaggggagactgacgtcatctactcgctcatcatccgccggaagccgctcttctacgtcattaacatcatcgtgccctgtgtgctcatctcgggcctggtgctgctcgcctacttcctgccggcgcaggccggcggccagaaatgcacggtctccatcaacgtcctgctcgcccagaccgtcttcttgttcctcattgcccagaaaatcccagagacttctctgagcgtgccgctcctgggcaggttccttattttcgtcatggtggtcgccacgctcattgtcatgaattgcgtcatcgtgctcaacgtgtcccagcggacgcccaccacccacgccatgtccccgcggctgcgccacgttctcctggagctgctgccgcgcctcctgggctccccgccgccgcccgaggccccccgggccgcctcgcccccaaggcgggcgtcgtcggtgggcttattgctccgcgcggaggagctgatactgaaaaagccacggagcgagctcgtgtttgaggggcagaggcaccggcaggggacctggacggctgccttctgccagagcctgggcgccgccgcccccgaggtccgctgctgtgtggatgccgtgaacttcgtggccgagagcacgagagatcaggaggccaccggcgaggaagtgtccgactgggtgcgcatggggaatgcccttgacaacatctgcttctgggccgctctggtgctcttcagcgtgggctccagcctcatcttcctcggggcctacttcaaccgagtgcctgatctcccctacgcgccgtgtatccagccttag

SEQ ID NO: 8 - protein, 493 aa, Homo sapiens
MARAPLGVLLLLGLLGRGVGKNEELRLYHHLFNNYDPGSRPVREPEDTVTISLKVTLTNLISLNEKEETLTTSVWIGIDWQDYRLNYSKDDFGGIETLRVPSELVWLPEIVLENNIDGQFGVAYDANVLVYEGGSVTWLPPAIYRSVCAVEVTYFPFDWQNCSLIFRSQTYNAEEVEFTFAVDNDGKTINKIDIDTEAYTENGEWAIDFCPGVIRRHHGGATDGPGETDVIYSLIIRRKPLFYVINIIVPCVLISGLVLLAYFLPAQAGGQKCTVSINVLLAQTVFLFLIAQKIPETSLSVPLLGRFLIFVMVVATLIVMNCVIVLNVSQRTPTTHAMSPRLRHVLLELLPRLLGSPPPPEAPRAASPPRRASSVGLLLRAEELILKKPRSELVFEGQRHRQGTWTAAFCQSLGAAAPEVRCCVDAVNFVAESTRDQEATGEEVSDWVRMGNALDNICFWAALVLFSVGSSLIFLGAYFNRVPDLPYAPCIQP

SEQ ID NO: 9 - DNA, 1554 bp, Homo sapiens
atgcatgggggccaggggccgctgctcctcctgctgctgctggctgtctgcctgggggcccagggccggaaccaggaggagcgcctgctcgcagacctgatgcaaaactacgaccccaacctgcggcccgcggaacgagactcggatgtggtcaatgtcagcctgaagctaaccctcaccaacctcatctccctgaacgagcgagaggaagccctcaccaccaatgtctggatagagatgcagtggtgcgactatcgcctgcgctgggatccgcgagactacgaaggcctgtgggtgctgagggtgccgtccaccatggtgtggcggccggatatcgtgctggagaacaacgtggacggtgtcttcgaggtggccctctactgcaatgtgctcgtgtcccctgacggctgtatctactggctgccgcctgccatcttccgttccgcctgctctatctcagtcacctacttccccttcgactggcagaactgctcccttatcttccagtcccagacttacagcaccaatgagattgatctgcagctgagtcaggaagatggccagaccatcgagtggattttcattgaccctgaggccttcacagagaatggggagtgggccatccagcaccgaccagccaagatgctcctggacccagcggcgccagcccaggaagcaggccaccagaaggtggtgttctacctgctcatccagcgcaagcccctcttctacgtcatcaacatcatcgccccctgtgtgctcatctcctctgtcgccatcctcatccacttccttcctgccaaggctgggggccagaagtgtaccgtcgccatcaacgtgctcctggcccagactgtcttcctcttccttgtggccaagaaggtgcctgaaacctcccaggcggtgccactcatcagcaagtacctgaccttcctcctggtggtgaccatcctcattgtcgtgaatgctgtggttgtgctcaatgtctccttgcggtctccacacacacactccatggcccgaggggtccgcaaggtgttcctgaggctcttgccccagctgctgaggatgcacgttcgcccgctggccccggcagctgtgcaggacacccagtcccggctacagaatggctcctcgggatggtcgatcacaactggggaggaggtggccctctgcctgcctcgcagtgaactcctcttccagcagtggcagcggcaagggctggtggcggcagcgctggagaagctagagaaaggcccggagttagggctgagccagttctgtggcagcctgaagcaggctgccccagccatccaggcctgtgtggaagcctgcaacctcattgcctgtgcccggcaccagcagagtcactttgacaatgggaatgaggagtggttcctggtgggccgagtgctggaccgcgtctgcttcctggccatgctctcgctcttcatctgtggcacagctggcatcttcctcatggcccactacaaccgggtgccggccctgccattccctggagatccacgcccctacctgccctcaccagactga

SEQ ID NO: 10 - protein, 517 aa, Homo sapiens
MHGGQGPLLLLLLLAVCLGAQGRNQEERLLADLMQNYDPNLRPAERDSDVVNVSLKLTLTNLISLNEREEALTTNVWIEMQWCDYRLRWDPRDYEGLWVLRVPSTMVWRPDIVLENNVDGVFEVALYCNVLVSPDGCIYWLPPAIFRSACSISVTYFPFDWQNCSLIFQSQTYSTNEIDLQLSQEDGQTIEWIFIDPEAFTENGEWAIQHRPAKMLLDPAAPAQEAGHQKVVFYLLIQRKPLFYVINIIAPCVLISSVAILIHFLPAKAGGQKCTVAINVLLAQTVFLFLVAKKVPETSQAVPLISKYLTFLLVVTILIVVNAVVVLNVSLRSPHTHSMARGVRKVFLRLLPQLLRMHVRPLAPAAVQDTQSRLQNGSSGWSITTGEEVALCLPRSELLFQQWQRQGLVAAALEKLEKGPELGLSQFCGSLKQAAPAIQACVEACNLIACARHQQSHFDNGNEEWFLVGRVLDRVCFLAMLSLFICGTAGIFLMAHYNRVPALPFPGDPRPYLPSPD

SEQ ID NO: 11 - DNA, 1515 bp, Homo sapiens
atgaccgaggcggcgctggtggagggccaggtcaagctgcgggacggcaagaagtggaagagtaggtggctggtgctgcggaagccgtcgcccgtggcagactgcctgctgatgctggtctacaaggacaagtcggagcgtatcaagggcctgcgggagcgcagcagcctgacgctagaggacatctgcgggctggagcccggcctgccctacgagggcctggtccacacgctggccattgtctgcctgtcccaggccatcatgctgggctttgacagccacgaggccatgtgtgcgtgggatgcccggatccgctatgcgctcggcgaggtgcataggttccatgtgacagtggctccaggcaccaagttggagagcggcccggctaccctgcacctctgcaatgatgtcctcgtcttggccagggacatccccccggctgtcacggggcagtggaagctgtctgacctccggcgctacggggccgtgccaagcggattcatctttgaaggcgggaccaggtgtgggtactgggctggcgtcttcttcctgtcctcggccgagggggagcagatcagcttcctgttcgactgcatcgtccgaggcatctcccccaccaagggcccctttgggctgcggccggttctaccagacccaagtcccccgggaccctcgactgtggaggagcgtgtggcccaggaagccctggaaaccctacagctggagaagcggctgagcctcctctcacatgcgggcaggccgggcagtggaggggatgaccgcagcctgtccagctcatcctcagaggccagtcacttggacgtcagcgccagcagccggctcaccgcatggccagagcaatcctcgtcgtcagccagcacgtcacaggaggggcctagaccagcagctgcccaggccgccggggaagccatggtgggtgcctcaaggccaccccccaagccgctgcgtccgcggcagctgcaggaggttggccgccagagctcctcggacagcggcatcgccactggcagccactcctcttactccagcagcctctcgtcctacgcgggcagcagcctggacgtgtggcgggccacagatgaactgggctcactgctcagcctgccagcagcgggggcccccgagcccagcctgtgcacctgcctgcccgggacagtcgagtaccaggtgcccacctccctgcgggcccactatgacacaccacgcagcctttgcctggctcctagagaccacagccccccctcacagggcagccccggcaacagtgcggccagggactcaggcggccagacgtccgccgggtgtccctctggctggctgggcacgagacggcggggcctggtgatggaggccccccagggcagcgaggccacactgcctggccctgcccctggcgagccctgggaagcaggcggcccccacgcggggccacccccggctttcttttcggcatgtccagtctgtggaggactcaaggtaaacccccctccttga

SEQ ID NO: 12 - protein, 504 aa, Homo sapiens
MTEAALVEGQVKLRDGKKWKSRWLVLRKPSPVADCLLMLVYKDKSERIKGLRERSSLTLEDICGLEPGLPYEGLVHTLAIVCLSQAIMLGFDSHEAMCAWDARIRYALGEVHRFHVTVAPGTKLESGPATLHLCNDVLVLARDIPPAVTGQWKLSDLRRYGAVPSGFIFEGGTRCGYWAGVFFLSSAEGEQISFLFDCIVRGISPTKGPFGLRPVLPDPSPPGPSTVEERVAQEALETLQLEKRLSLLSHAGRPGSGGDDRSLSSSSSEASHLDVSASSRLTAWPEQSSSSASTSQEGPRPAAAQAAGEAMVGASRPPPKPLRPRQLQEVGRQSSSDSGIATGSHSSYSSSLSSYAGSSLDVWRATDELGSLLSLPAAGAPEPSLCTCLPGTVEYQVPTSLRAHYDTPRSLCLAPRDHSPPSQGSPGNSAARDSGGQTSAGCPSGWLGTRRRGLVMEAPQGSEATLPGPAPGEPWEAGGPHAGPPPAFFSACPVCGGLKVNPPP